European Patent Application EP 4 733 394 A1, published April 29, 2026. Title: REVERSE TRANSCRIPTASE ENZYMES, COMBINATIONS, METHODS, AND USES THEREOF. Applicant: NZYTECH LDA. Application EP P1722.3 EP, filed February 5, 2025. The sequence listing filed with the application follows.

SEQUENCE LISTING (15 sequences)

SEQ ID NO: 1 - protein, 522 aa, Moloney Murine Leukemia Virus
MGSSHHHHHHSSGLVPRGSHMASTWLSDFPQAWAETGGMGLAVRQAPLIIPLKATSTPVSIKQYPMSQEARLGIKPHIQRLLDQGILVPCQSPWNTPLLPVKKPGTNDYRPVQDLREVNKRVEDIHPTVPNPYNLLSGLPPSHQWYTVLDLKDAFFCLRLHPTSQPLFAFEWRDPEMGISGQLTWTRLPQGFKNSPTLFDEALHRDLADFRIQHPDLILLQYVDDLLLAATSELDCQQGTRALLQTLGNLGYRASAKKAQICQKQVKYLGYLLKEGQRWLTEARKETVMGQPTPKTPRQLREFLGTAGFCRLWIPGFAEMAAPLYPLTKTGTLFNWGPDQQKAYQEIKQALLTAPALGLPDLTKPFELFVDEKQGYAKGVLTQKLGPWRRPVAYLSKKLDPVAAGWPPCLRMVAAIAVLTKDAGKLTMGQPLVILAPHAVEALVKQPPDRWLSNARMTHYQALLLDTDRVQFGPVVALNPATLLPLPEEGLQHNCLDILAEAHGTRPDLTDQPLLEHHHHHH

SEQ ID NO: 2 - protein, 522 aa, synthetic construct
MGSSHHHHHHSSGLVPRGSHMASTWLSDFPQAWAETGGMGLAVRQAPVVVELKSDASPVAVRQYPMSREAQEGIRPHIQRFLDLGVLVPCQSPWNTPLLPVKKPGTNDYRPVQDLREVNKRVQDIHPTVPNPYNLLSSLPPSHTWYTVLDLKDAFFCLKLHPNSQPLFAFEWRDPEKGHTGQLTWTRLPQGFKNSPTLFDEALHRDLASFRASNPQVVLLQYVDDLLVAAPTYEDCKEGTQKLLQELSNLGYRVSAKKAQLCQKEVTYLGYLLKEGQRWLTPARKATVMGIPTPTTPRQVREFLGTAGFCRLWIPGFASLAAPLYPLTKESTPFLWTEEHQKAFDCIKEALLTAPALALPDLTKPFALYVDERDGVARGVLTQTLGPWRRPVAYLSKKLDPVASGWPTCLKAVAAVALLLKDADKLTLGQNVTVIASHSLESIVRQPPDRWMSKARMTHYQALLLDTDRVQFGPVVALNPATLLPLPEEGLQHNCLDILAEAHGTRPDLTDQPLLEHHHHHH

SEQ ID NO: 3 - protein, 696 aa, synthetic construct
MGSSHHHHHHSSGPQQGLRTLNIEDEHRLHETSKEPDVSLGSTWLSDFPQAWAETGGMGLAVRQAPVVVELKSDASPVAVRQYPMSREAQEGIRPHIQRFLDLGVLVPCQSPWNTPLLPVKKPGTNDYRPVQDLREVNKRVQDIHPTVPNPYNLLSSLPPSHTWYTVLDLKDAFFCLKLHPNSQPLFAFEWRDPEKGHTGQLTWTRLPQGFKNSPTLFDEALHRDLASFRASNPQVVLLQYVDDLLVAAPTYEDCKEGTQKLLQELSNLGYRVSAKKAQLCQKEVTYLGYLLKEGQRWLTPARKATVMGIPTPTTPRQVREFLGTAGFCRLWIPGFASLAAPLYPLTKESTPFLWTEEHQKAFDCIKEALLTAPALALPDLTKPFALYVDERDGVARGVLTQTLGPWRRPVAYLSKKLDPVASGWPTCLKAVAAVALLLKDADKLTLGQNVTVIASHSLESIVRQPPDRWMSKARMTHYQALLLDTDRVQFGPVVALNPATLLPLPEEGLQHNCLDILAEAHGTRPDLTDQPLPDADHTWYTGGSSLLQEGQRKAGAAVTTETEVIWAKALPAGTSAQRAQLIALTQALKMAEGKKLNVYTNSRYAFATAHIHGEIYRRRGLLTSEGKEIKNKDEILALLKALFLPKRLSIIHCPGHQKGHSAEARGNRMADQAARKAAITETPDTSTLLIENSSP

SEQ ID NO: 4 - DNA, 20 bp, synthetic construct
  source 1..20: mol_type = other DNA
caaacacaaacggttcccag

SEQ ID NO: 5 - DNA, 20 bp, synthetic construct
  source 1..20: mol_type = other DNA
ttcaccttcccaaagaccac

SEQ ID NO: 6 - DNA, 22 bp, synthetic construct
  source 1..22: mol_type = other DNA
tgcttgccatccagccattcag

SEQ ID NO: 7 - DNA, 22 bp, synthetic construct
  source 1..22: mol_type = other DNA
tccaagatcaagtcctttgtga

SEQ ID NO: 8 - DNA, 20 bp, synthetic construct
  source 1..20: mol_type = other DNA
gtccctgaacacatccttgt

SEQ ID NO: 9 - DNA, 24 bp, synthetic construct
  source 1..24: mol_type = other DNA
actacaaccacctcatgcccacaa

SEQ ID NO: 10 - DNA, 38 bp, synthetic construct
  source 1..38: mol_type = other DNA
agcggtgaaccaagacgcagggcgcgatcaaaacaacg

SEQ ID NO: 11 - DNA, 41 bp, synthetic construct
  source 1..41: mol_type = other DNA
aattccctcgaggacaaggcgagctcttcggtagtagccaa

SEQ ID NO: 12 - DNA, 20 bp, synthetic construct
  source 1..20: mol_type = other DNA
ccagaatggagaacgcagtg

SEQ ID NO: 13 - DNA, 18 bp, synthetic construct
  source 1..18: mol_type = other DNA
ccgtcaccaccacgaatt

SEQ ID NO: 14 - DNA, 21 bp, synthetic construct
  source 1..21: mol_type = other DNA
ttattgggtaaaccttggggc

SEQ ID NO: 15 - DNA, 25 bp, synthetic construct
  source 1..25: mol_type = other DNA
ttccaattaacaccaatagcagtcc